European Patent Application EP 4 799 638 A1, published September 2, 2026. Title: 免疫佐剂组合物及其制备方法和用途. Applicant: 远大赛威信生命科学（南京）有限公司. The sequence listing filed with the application follows.

SEQUENCE LISTING (16 sequences)

SEQ ID NO: 1 - DNA, 21 bp, artificial sequence
  source 1..21: mol_type = other DNA
tcgttcgttcgttcgttcgtt

SEQ ID NO: 2 - DNA, 25 bp, artificial sequence
  source 1..25: mol_type = other DNA
tcgttcgttcgttcgttcgttcgtt

SEQ ID NO: 3 - DNA, 21 bp, artificial sequence
  source 1..21: mol_type = other DNA
tcgtcgtcgtcgtcgtcgtcg

SEQ ID NO: 4 - DNA, 22 bp, artificial sequence
  source 1..22: mol_type = other DNA
tgactgtgaacgttcgagatga

SEQ ID NO: 5 - DNA, 24 bp, artificial sequence
  source 1..24: mol_type = other DNA
tcgtcgttttgtcgttttgtcgtt

SEQ ID NO: 6 - DNA, 20 bp, artificial sequence
  source 1..20: mol_type = other DNA
tccatgacgttcctgacgtt

SEQ ID NO: 7 - DNA, 23 bp, artificial sequence
  source 1..23: mol_type = other DNA
tcgacgttcgtcgttcgtcgttc

SEQ ID NO: 8 - DNA, 20 bp, artificial sequence
  source 1..20: mol_type = other DNA
tccatgacgttcctgatgct

SEQ ID NO: 9 - DNA, 27 bp, artificial sequence
  source 1..27: mol_type = other DNA
tgtcgtcgtcgtttgtcgtttgtcgtt

SEQ ID NO: 10 - DNA, 20 bp, artificial sequence
  source 1..20: mol_type = other DNA
gggggacgatcgtcgggggg

SEQ ID NO: 11 - DNA, 21 bp, artificial sequence
  source 1..21: mol_type = other DNA
ggggacgacgtcgtggggggg

SEQ ID NO: 12 - DNA, 20 bp, artificial sequence
  source 1..20: mol_type = other DNA
tcgtcgtttcgcgcgcgccg

SEQ ID NO: 13 - DNA, 30 bp, artificial sequence
  source 1..30: mol_type = other DNA
tcgtcgttcgttcgtcgaacgacgtttgat

SEQ ID NO: 14 - protein, 678 aa, Hepatitis B virus
METGLUASNILETHRSERGLYPHELEUGLYPROLEULEUVALLEUGLNALAGLYPHEPHELEULEUTHRARGILELEUTHRILEPROGLNSERLEUASPSERTRPTRPTHRSERLEUASNPHELEUGLYGLYSERPROVALCYSLEUGLYGLNASNSERGLNSERPROTHRSERASNHISSERPROTHRSERCYSPROPROILECYSPROGLYTYRARGTRPMETCYSLEUARGARGPHEILEILEPHELEUPHEILELEULEULEUCYSLEUILEPHELEULEUVALLEULEUASPTYRGLNGLYMETLEUPROVALCYSPROLEUILEPROGLYSERTHRTHRTHRSERTHRGLYPROCYSLYSTHRCYSTHRTHRPROALAGLNGLYASNSERMETPHEPROSERCYSCYSCYSTHRLYSPROTHRASPGLYASNCYSTHRCYSILEPROILEPROSERSERTRPALAPHEALALYSTYRLEUTRPGLUTRPALASERVALARGPHESERTRPLEUSERLEULEUVALPROPHEVALGLNTRPPHEVALGLYLEUSERPROTHRVALTRPLEUSERALAILETRPMETMETTRPTYRTRPGLYPROSERLEUTYRSERILEVALSERPROPHEILEPROLEULEUPROILEPHEPHECYSLEUTRPVALTYRILE

SEQ ID NO: 15 - protein, 549 aa, Hepatitis B virus
METASPILEASPPROTYRLYSGLUPHEGLYALASERVALGLULEULEUSERPHELEUPROSERASPPHEPHEPROSERILEARGASPLEULEUASPTHRALASERALALEUTYRARGGLUALALEUGLUSERPROGLUHISCYSSERPROHISHISTHRALALEUARGGINALAILELEUCYSTRPGLYGLULEUMETASNLEUALATHRTRPVALGLYSERASNLEUGLUASPPROALASERARGGLULEUVALVALSERTYRVALASNVALASNMETGLYLEULYSILEARGGINLEULEUTRPPHEHISILESERCYSLEUTHRPHEGLYARGGLUTHRVALLEUGLUTYRLEUVALSERPHEGLYVALTRPILEARGTHRPROPROALATYRARGPROPROASNALAPROILELEUSERTHRLEUPROGLUTHRTHRVALVALARGARGARGGLYARGSERPROARGARGARGTHRPROSERPROARGARGARGARGSERGINSERPROARGARGARGARGSERGINSERARGGLUSERGINCYS

SEQ ID NO: 16 - protein, 1554 aa, artificial sequence
SERVALLEUARGTYRASPASPPHEHISILEASPGLUASPLYSLEUASPTHRASNSERVALTYRGLUPROTYRTYRHISSERASPHISALAGLUSERSERTRPVALASNARGGLYGLUSERSERARGLYSALATYRASPHISASNSERPROTYRILETRPPROARGASNASPTYRASPGLYPHELEUGLUASNALAHISGLUHISHISGLYVALTYRASNGINGLYARGGLYILEASPSERGLYGLUARGLEUMETGLNPROTHRGINMETSERALAGINGLUASPLEUGLYASPASPTHRGLYILEHISVALILEPROTHRLEUASNGLYASPASPARGHISLYSILEVALASNVALASPGINARGGLNTYRGLYASPVALPHELYSGLYASPLEUASNPROLYSPROGLNGLYGLNARGLEUILEGLUVALSERVALGLUGLUASNHISPROPHETHRLEUARGALAPROILEGLNARGILETYRGLYVALARGTYRTHRGLUTHRTRPSERPHELEUPROSERLEUTHRCYSTHRGLYASPALAALAPROALAILEGLNHISILECYSLEULYSHISTHRTHRCYSPHEGINASPVALVALVALASPVALASPCYSALAGLUASNTHRLYSGLUASPGINLEUALAGLUILESERTYRARGPHEGLNGLYLYSLYSGLUALAASPGLNPROTRPILEVALVALASNTHRSERTHRLEUPHEASPGLULEUGLULEUASPPROPROGLUILEGLUPROGLYVALLEULYSVALLEUARGTHRGLULYSGINTYRLEUGLYVALTYRILETRPASNMETARGGLYSERASPGLYTHRSERTHRTYRALATHRPHELEUVALTHRTRPLYSGLYASPGLULYSTHRARGASNPROTHRPROALAVALTHRPROGLNPROARGGLYALAGLUPHEHISMETTRPASNTYRHISSERHISVALPHESERVALGLYASPTHRPHESERLEUALAMETHISLEUGLNTYRLYSILEHISGLUALAPROPHEASPLEULEULEUGLUTRPLEUTYRVALPROILEASPPROTHRCYSGINPROMETARGLEUTYRSERTHRCYSLEUTYRHISPROASNALAPROGINCYSLEUSERHISMETASNSERGLYCYSTHRPHETHRSERPROHISLEUALAGLNARGVALALASERTHRVALTYRGLNASNCYSGLUHISALAASPASNTYRTHRALATYRCYSLEUGLYILESERHISMETGLUPROSERPHEGLYLEUILELEUHISASPGLYGLYTHRTHRLEULYSPHEVALASPTHRPROGLUSERLEUSERGLYLEUTYRVALPHEVALVALTYRPHEASNGLYHISVALGLUALAVALALATYRTHRVALVALSERTHRVALASPHISPHEVALASNALAILEGLUGLUARGGLYPHEPROPROTHRALAGLYGLNPROPROALATHRTHRLYSPROLYSGLUILETHRPROVALASNPROGLYTHRSERPROLEULEUARGGLYGLYGLYGLYSERHISHISHISHISHISHIS